European Patent Application EP 4 488 225 A1, published January 8, 2025. Title: METHOD FOR PRODUCING PHOSPHORIC ACID. Applicant: KINKI UNIVERSITY. Application WO PCT/JP2023/007246, filed February 28, 2023. The sequence listing filed with the application follows.

SEQUENCE LISTING (23 sequences)

SEQ ID NO: 1 - DNA, 19 bp, synthetic construct
  misc_feature 1..19: note = Primer_ACT_F
  source 1..19: mol_type = other DNA
gcatcacactttctacaac

SEQ ID NO: 2 - DNA, 19 bp, synthetic construct
  misc_feature 1..19: note = Primer_ACT_R
  source 1..19: mol_type = other DNA
cctggatagcaacatacat

SEQ ID NO: 3 - DNA, 20 bp, synthetic construct
  misc_feature 1..20: note = Primer_GSTU19_F
  source 1..20: mol_type = other DNA
actgaacatagataggaacc

SEQ ID NO: 4 - DNA, 19 bp, synthetic construct
  misc_feature 1..19: note = Primer_GSTU19_R
  source 1..19: mol_type = other DNA
gtggacattggattgattg

SEQ ID NO: 5 - DNA, 20 bp, synthetic construct
  misc_feature 1..20: note = Primer_CAT2_F
  source 1..20: mol_type = other DNA
gggcaataagcaaatatgaa

SEQ ID NO: 6 - DNA, 19 bp, synthetic construct
  misc_feature 1..19: note = Primer_CAT2_R
  source 1..19: mol_type = other DNA
gcaacctggagatagatac

SEQ ID NO: 7 - DNA, 18 bp, synthetic construct
  misc_feature 1..18: note = Primer_LAX2-1_F
  source 1..18: mol_type = other DNA
gtgggagaaagtgatagg

SEQ ID NO: 8 - DNA, 18 bp, synthetic construct
  misc_feature 1..18: note = Primer_LAX2-1_R
  source 1..18: mol_type = other DNA
attgattggaccgaagaa

SEQ ID NO: 9 - DNA, 22 bp, synthetic construct
  misc_feature 1..22: note = Primer_GST12_F
  source 1..22: mol_type = other DNA
ggatggaataatgaatgaatga

SEQ ID NO: 10 - DNA, 18 bp, synthetic construct
  misc_feature 1..18: note = Primer_GST12_R
  source 1..18: mol_type = other DNA
agttttggcacatacagt

SEQ ID NO: 11 - DNA, 18 bp, synthetic construct
  misc_feature 1..18: note = Primer_CaM5_F
  source 1..18: mol_type = other DNA
caaagaacccatcacaga

SEQ ID NO: 12 - DNA, 18 bp, synthetic construct
  misc_feature 1..18: note = Primer_CaM5_R
  source 1..18: mol_type = other DNA
aacagaggaagaggacat

SEQ ID NO: 13 - protein, 7 aa, unidentified
GIAGPPG

SEQ ID NO: 14 - protein, 11 aa, unidentified
AGLPGVAGAPG

SEQ ID NO: 15 - protein, 14 aa, unidentified
PGAPGPKGELGPVG

SEQ ID NO: 16 - protein, 11 aa, unidentified
DVPAASLVVGP

SEQ ID NO: 17 - protein, 12 aa, unidentified
AGADAGATPVVD

SEQ ID NO: 18 - protein, 14 aa, unidentified
AQPSIPAADGSVPV

SEQ ID NO: 19 - protein, 12 aa, unidentified
SALRPDGEYTLL

SEQ ID NO: 20 - protein, 10 aa, unidentified
GCPAVLPIDH

SEQ ID NO: 21 - protein, 10 aa, unidentified
KDLPETLNEL

SEQ ID NO: 22 - protein, 11 aa, unidentified
GIKEQDIDKDL

SEQ ID NO: 23 - protein, 10 aa, unidentified
DQHPIDGYLS